European Patent Specification EP 3 493 812 B1, published January 4, 2023. Title: COMBINATION TREATMENT FOR HEMATOLOGICAL CANCERS. Applicant: JANSSEN BIOTECH, INC. The sequence listing filed with the application follows.

SEQUENCE LISTING (8 sequences)

SEQ ID NO: 1 - DNA, 13 bp, Artificial Sequence
  source: /note="Description of Artificial Sequence: Synthetic oligonucleotide"
tagggttagacaa

SEQ ID NO: 2 - DNA, 13 bp, Artificial Sequence
  source: /note="Description of Artificial Sequence: Synthetic oligonucleotide"
taggtgtaagcaa

SEQ ID NO: 3 - DNA, 13 bp, Artificial Sequence
  source: /note="Description of Artificial Sequence: Synthetic oligonucleotide"
aacagattgggat

SEQ ID NO: 4 - DNA, 24 bp, Artificial Sequence
  source: /note="Description of Artificial Sequence: Synthetic primer"
tgtactttgtcaaggtggatgtga

SEQ ID NO: 5 - DNA, 23 bp, Artificial Sequence
  source: /note="Description of Artificial Sequence: Synthetic primer"
gctggaggtctgtcaaggtagag

SEQ ID NO: 6 - DNA, 15 bp, Artificial Sequence
  source: /note="Description of Artificial Sequence: Synthetic probe"
cgcgtacgacaccat

SEQ ID NO: 7 - DNA, 18 bp, Artificial Sequence
  source: /note="Description of Artificial Sequence: Synthetic primer"
aatccgtcgagcagagtt

SEQ ID NO: 8 - DNA, 30 bp, Artificial Sequence
  source: /note="Description of Artificial Sequence: Synthetic primer"
gcgcggcttacccttacccttaccctaacc